European Patent Specification EP 3 690 042 B1, published May 6, 2026. Title: Parthenocarpy regulatory gene and Use thereof. Applicant: NATIONAL RESEARCH AND DEVELOPMENT AGENCY NATIONAL AGRICULTURE AND FOOD RESEARCH ORGANIZATION, TAKII & CO., LTD. The sequence listing filed with the application follows.

SEQUENCE LISTING (78 sequences)

SEQ ID NO: 1 - protein, 394 aa, Solanum melongena
MGSFGMLARRAVLTDTPVMVQIQELIRGNKDCISLAQGVVYWQPPAQALEKVKEIIWEPSVSRYGADEGLPELREALMQKLGHENNLHKSSVMVTAGANQAFVNVVLTLCDAGDSVVMFAPYYFNAHMSFQMTGVTDILVGPGDPKTLHPDADWLESTLKNTVPTPKLVTVVNPGNPSGTYIPESLLKRISDICKKAGCWLVIDNTYEYFMYDNRKHVCIEANHIVNIFSFSKAYGMMGWRVGYIAYPSEVEGLAAQLLKVQDNIPICASIISQRLALYSMEMGPEWVTNQVKDLVKNREVLLEALSPLGKGAVKGGEGAIYLWAKLPDKYMDDFKVVHWLAKRHGVVLIPGSSSGCPGYVRVSFGGLIEKDCRAAAERLRKGLEELVNSGMAS

SEQ ID NO: 2 - DNA, 1625 bp, Solanum melongena
gtccgtagcagtcaaatttattcatatttaacaaaaagatccaatttttatattttttacaatccctttatataggttccaagctttttgtaagattttcagaaagggaaaggccttttttgctctgtgggtaggtggataagaactcttttcttgaaggtagtgtttattttattgtttttactgagaaagaggaaatgggttctttcggaatgctcgctagaagagctgttcttaccgatacaccagttatggttcagatacaagaactgattcgaggtaataaagattgtatttctctagctcagggagtagtgtactggcaaccacctgcacaagcacttgaaaaggtgaaagaaattatctgggaaccttcagttagtcgctatggtgctgatgagggccttcctgagcttagggaggcgttgatgcaaaagttgggtcatgaaaataacctccataaatcctcggtgatggttactgctggtgctaatcaggctttcgtaaatgtcgttctcaccctgtgtgatgctggtgattcagttgttatgtttgcaccatactatttcaatgcacacatgtcattccagatgacaggtgttactgatattctggtgggtcctggtgatcccaagacactccatcctgatgcagactggttggagagtactttaaagaatactgtaccaacaccaaagctcgtcactgttgttaatcctggcaatccatcaggaacatatatccccgagtctcttcttaagaggatatctgatatttgtaagaaggcaggatgttggctcgtaattgataacacatatgagtatttcatgtatgataatcggaaacatgtttgcatagaagcaaaccacattgtcaacatcttttccttctctaaagcatatgggatgatgggatggagagttggatatatagcatacccatcggaagtggaagggcttgcagctcaactccttaaagttcaggacaacataccaatctgtgcttcaataatctcacaacgactggctctttactcaatggaaatgggaccagaatgggtaactaatcaagtaaaagaccttgtcaagaacagagaggtgcttctagaagccttatctcctttgggaaagggagctgttaaagggggagaaggtgccatttacctgtgggcaaagctgccagataaatacatggacgacttcaaagtagttcactggctagctaagaggcatggagtagtcctgatccctggaagttccagcggttgtccaggttatgttagggtctcctttggaggattgatcgagaaggactgtcgagcagctgcagaaaggctcagaaaaggtttggaagagctggtaaatagtggaatggcgtcatgattctctctgactaaaatttagtgtcagctggttctcctggacatcagtcatcaacaatacaatgacagacactttctatccttaataattgaagggttttaagctttgcaacttgatcattggacatgcaagttaaaacttgccattctgtatagtttgaaatgaagtattcatagatacctacttttcttaaatggatgatggaagtgtctcatttatctcagagcatatctcattgaatca

SEQ ID NO: 3 - DNA, 1305 bp, Solanum melongena
tttttgctctgtgggtaggtggataagaactcttttcttgaaggtagtgtttattttattgtttttactgagaaagaggaaatgggttctttcggaatgctcgctagaagagctgttcttaccgatacaccagttatggttcagatacaagaactgattcgaggtaataaagattgtatttctctagctcagggagtagtgtactggcaaccacctgcacaagcacttgaaaaggtgaaagaaattatctgggaaccttcagttagtcgctatggtgctgatgagggccttcctgagcttagggaggcgttgatgcaaaagttgggtcatgaaaataacctccataaatcctcggtgatggttactgctggtgctaatcaggctttcgtaaatgtcgttctcaccctgtgtgatgctggtgattcagttgttatgtttgcaccatactatttcaatgcacacatgtcattccagatgacaggtgttactgatattctggtgggtcctggtgatcccaagacactccatcctgatgcagactggttggagagtactttaaagaatactgtaccaacaccaaagctcgtcactgttgttaatcctggcaatccatcaggaacatatatccccgagtctcttcttaagaggatatctgatatttgtaagaaggcaggatgttggctcgtaattgataacacatatgagtatttcatgtatgataatcggaaacatgtttgcatagaagcaaaccacattgtcaacatcttttccttctctaaagcatatgggatgatgggatggagagttggatatatagcatacccatcggaagtggaagggcttgcagctcaactccttaaagttcaggacaacataccaatctgtgcttcaataatctcacaacgactggctctttactcaatggaaatgggaccagaatgggtaactaatcaagtaaaagaccttgtcaagaacagagaggtgcttctagaagccttatctcctttgggaaagggagctgttaaagggggagaaggtgccatttacctgtgggcaaagctgccagataaatacatggacgacttcaaagtagttcactggctagctaagaggcatggagtagtcctgatccctggaagttccagcggttgtccaggttatgttagggtctcctttggaggattgatcgagaaggactgtcgagcagctgcagaaaggctcagaaaaggtttggaagagctggtaaatagtggaatggcgtcatgattctctctgactaaaatttagtgtcagctggttctcctg

SEQ ID NO: 4 - DNA, 6528 bp, Solanum melongena
gtccgtagcagtcaaatttattcatatttaacaaaaagatccaatttttatattttttacaatccctttatataggttccaagctttttgtaagattttcagaaagggaaaggccttttttgctctgtgggtaggtggataagaactcttttcttgaaggtagtgtttattttattgtttttactgagaaagaggaaatgggttctttcggaatgctcgctagaagagctgttcttaccgatacaccagttatggttcaggtaaattacaagatcctagattggatttcttgctcttttgtttggtttaaggttctgtgctttaatgggatatgttgttgttgtgttttgcaatcgatagatacaagaactgattcgaggtaataaagattgtatttctctagctcaggtttgtttactttctccaatgtttgtttcattttgttttactatatcttagttttattattctacttttcattgaatggttcaaaaagttgagaactttgataaaattcatctgttgttgtgatgtctttgaagcctacatatcatcttattgtgcctttcgaaatcttgattagattgacttacattaaaaattggctaattcattcttgaagttatcaatttcaattttttttttcagttgaaatatgaattgcttaatatttaagctagtaattggggaaaaaaaatcaaactggacttccctcccatgtaaagaatgtatttgcagatggttttgaatgtgaaaaatggagattatgagtgtccactgagctgggtgggtataagggcttgggtaggtgggtttcgggcctagagcacatgtgaaggaggtctactggtacaagattgacattttctctttccttaagttcctctggtgattgcaaataacataaattgcctgagcttcttgttttgcgaagaaatcttctgaggtttctcccatgatctctggagttacaaaattattttgctagtatgttccatgctcggttgtccttttcctgtgcaaaaagagttataatactgttcttttgatctgtttttatttgggttaaccaagtatgatgtgatacagaagaatatctgccgccctaccatgtgctgtgagtagtgatccctttgtgttatcctcctattattggactgttttacgaatgactggttctattatgatctctgaggactgatctgttgacaagcaagttttatcaacctccatctgaaaaaaaagaaagtttaatcaacctaaacctaccaatggaagttttagaagttgtatagtttgctggggttggggcctggggaatgagtgtgtacttatttgcttctttatgtaccttccagagagagtaaacaaaggaatagagttatctgttgttggtggatctttctgttgaagtgtgtagttatattggttttgcctgaatatggttgtccatgttttccatccatgtatcttggtaccatcttatttttttctccgtcttacagggagtagtgtactggcaaccacctgcacaagcacttgaaaaggtgaaagaaattatctgggaaccttcagttagtcgctatggtgctgatgagggccttcctgagcttagggaggcgttgatgcaaaaggtatggtctatcagctggattactctaatactctggttttcatcgtatgggctgggtagtggaacaaacattggagtggtgtagggtgcttttgccaggtgaaacggtagttactgtcatgtatgaagttggattcatttcatgttttcaaactatatcattcacttgttgagttttggtttttacgttgtttggtctaatactttctttgtgctcttctccagttgggtcatgaaaataacctccataaatcctcggtgatggttactgctggtgctaatcaggtaaaatgttacttttttactattcagtcatctgaggatatagggtcagtcacttcacctctttttcttacctgccctgaatagtagtaggctacctttctttctcgcctttcttccatctttttccagataaaggttggatgttttagaatgaaactgcgttttggagatttgtttgcttgagttagagtgggttgagattgattctaccttcatacaagattcatttgctttgacagaggaccagtatttgggtgcatgtttacttcaccttcctaagctattcttcagttccccttttcccttcattaatgttcaaagttgtctagttcatactagaaacacggcagggctcctcttaaaaaaagaaagtgcaattttctactttttgcattgtcacaatactaagagatttcatctccaaaaccaggaagtgatgcttgtgagggaacgttttccctttctttttacccctctctctatctctctcttaaatgaagatttcttagagtttatgtggtcaagaaaccgtacagtacttttcctgataaatggtatggatacttctgaaagaaaaatagaactgcctcactgataaatggtgtgggattccactaggtatgttgttgttgttgttgttttctctatcatgatgcatacagtatgcagtgtatggaaaggttggtgtgattttgagatttggattttattttcttctgcttctacccatctaaagattattctttttctcgtgtgtatttttcttgataaaaaagatcattcttctgttgtgggcttattcagctccatgttctaacttgatcaaaaaagtcaaatgtgctctctttttcttgtcttttccgttttttgtaataagacctcttttagtttttgcatgttatcactgtacttttgtatgttaccattttcatgagatgacaatcttgcaatgggaacatatgcagcacaaaactctccatttagtatcatctgtcagaaacatatagggaaagaatctactgacatatctagcatgctcaagcacttggccctcacaattttgtctgcaaaatggaacttagggattacttcgactactaatttgagaattaattgcctagattttcaatgactgagtaaatgatggtccaaggggctcagaaagtatgagtacagacacatcattacgtacctgtccattacagagcagtattctctttttgaacaggagaattgtgtcctcaatagtcctccaaattaaaatcacaatttattgcaataaacaaattcggatgaaaccttaagctgaatgaagatagtagagctatgttaatgagccatttgtagagcaatagagttgctacatgtatgggtaaattaattagtgtattgtctatattctttgttagtgactaatggactagctgtatccctatcacttagaaatcactaatggagtctcactgaattgattccaggctttcgtaaatgtcgttctcaccctgtgtgatgctggtgattcagttgttatgtttgcaccatactatttcaatgcacacatgtcattccagatgacaggtgttactgatattctggtgggtcctggtgatcccaagacactccatcctgatgcaggtttgtaagttcagatgatgttcattttgtgataccctccccattattaagactgctattcctttagtttccttaagactgattacactagatgttgtcatatacatctctgttgtgtagcatgcatgttcaagtttgagggaacatcctttttatctttgtcatctcagcactttggaatatatatcataatcactaatcacatatgtactatgagttacttttttcctctttgcttgaaatttatcaaaaaactccatcttctctgaatctaacactacttgtgcagaaatcaacttaagaagaggttgctgcagaagtagtgttcagctttgtattgcaagttgtgtaaatcattcataatggtctattagtcttgatttgtagaatgttgtctggaaagcaatcattctgtgttttttctcgtattggatgtcctcaccccatccccaccagaaagaaaccaaaaaaaataatgaatttagtaaacttatagtttgacactttgaagcataatgttaacctaaatattgcttctattttgcataatggacttgagagtttcaaaacattatctgccttcgttatttgattgtttatggattgatatattccatgatttctcaattttcagactggttggagagtactttaaagaatactgtaccaacaccaaagctcgtcactgttgttaatcctggcaatccatcaggaacatatatccccgagtctcttcttaaggtctctatctcatctttatagatatgaatgtattggttgaagtcatcagttattcaaagtgcattactattctcatctgatttttactttattgaaacatcaacaagttgcattttgttcatgtagaggatatctgatatttgtaagaaggcaggatgttggctcgtaattgataacacatatgagtaagttactttttctgttgcatacgaatcttttagtttctcattttaaattgtgtactggttgttaataactggtgccgatatgttttctcatccatggatgaaagatgacattcttagaactaaagatgatgagggttgttgaatggactaatcctggaatacttttggttagaccagcaagagattattgaataaaccaaggaaacaggtcgtttgcattgcattgtgaggaaatctttttgctttgtgaacctaaacttgaactaaatttgataggcaagaaaatttatggtatcctgggatctgttgccatattttgattgctgagaaggggagaaaggaaatagctaaggtgaaagaatgatcagtctttgaattcatccaaattggcccacttgttgctgtttgttctcaatctctagatggaaaataagcctagaaagttggcttctcaacgagttagatagttaggacacattactattgagtctttcctcctccatgaatgtgaacatcttgttctgtcaaacatcatctctgttccttctttttcttgcaactttttgctttacactctgcttgtcgttttctatattcctgaatgatatgttcttatatatatgttgtaagttatttgcaggtatttcatgtatgataatcggaaacatgtttgcatagaagcaaaccacattgtcaacatcttttccttctctaaagcatatgggatgatgggatggagagttggatatgtaagtgatgcttgttctaacttatatctagcaatgtaataatattgggcagacaagtgattattattctgctgggtgagcctcaacacaaccagaaaatatacctggttaaaagatgattttttctatgttttccgcaactgcatcttcttgcctcataaactccctcgtctttacctttaaaccaaaaaccaaaaaaaatttaaaaaaattaaactgttgtctttacttatacctctttttaaaaccagcatgtatgacacctttaatcagtctctctatccttgtccatcattaacttttataacgaataatgttgcgtcctgtcatttgtgcctggttgagtgatctgctggaattggatataaaattggcctcaataacaaccaaaatacaagtgttcttttgcaacaaaaaggagttgttccaacagctaagacttatggcatatgagacatgattgctttaccagatgtttttgctgcaatgtaaattttgcagcaaaattcctcagcaaacttttgtactgaagatttactcctgaatggagaaggttgtttcatcttgtgagtgagctaaactcatgtcttaatcgatgcagatagcatacccatcggaagtggaagggcttgcagctcaactccttaaagttcaggacaacataccaatctgtgcttcaataatctcacaacgactggctctttactcaatggaaatgggaccagaatgggtaactaatcaagtaaaagaccttgtcaagaacagagaggtgcttctagaagccttatctcctttgggaaagggagctgttaaagggggagaaggtgccatttacctgtgggcaaagctgccagataaatacatggacgacttcaaagtagttcactggctagctaagaggcatggagtagtcctgatccctggaagttccagcggttgtccaggttatgttagggtctcctttggaggattgatcgagaaggactgtcgagcagctgcagaaaggctcagaaaaggtttggaagagctggtaaatagtggaatggcgtcatgattctctctgactaaaatttagtgtcagctggttctcctggacatcagtcatcaacaatacaatgacagacactttctatccttaataattgaagggttttaagctttgcaacttgatcattggacatgcaagttaaaacttgccattctgtatagtttgaaatgaagtattcatagatacctacttttcttaaatggatgatggaagtgtctcatttatctcagagcatatctcattgaatca

SEQ ID NO: 5 - DNA, 260 bp, Solanum melongena
gtccgtagcagtcaaatttattcatatttaacaaaaagatccaatttttatattttttacaatccctttatataggttccaagctttttgtaagattttcagaaagggaaaggccttttttgctctgtgggtaggtggataagaactcttttcttgaaggtagtgtttattttattgtttttactgagaaagaggaaatgggttctttcggaatgctcgctagaagagctgttcttaccgatacaccagttatggttcag

SEQ ID NO: 6 - DNA, 100 bp, Solanum melongena
gtaaattacaagatcctagattggatttcttgctcttttgtttggtttaaggttctgtgctttaatgggatatgttgttgttgtgttttgcaatcgatag

SEQ ID NO: 7 - DNA, 48 bp, Solanum melongena
atacaagaactgattcgaggtaataaagattgtatttctctagctcag

SEQ ID NO: 8 - DNA, 1097 bp, Solanum melongena
gtttgtttactttctccaatgtttgtttcattttgttttactatatcttagttttattattctacttttcattgaatggttcaaaaagttgagaactttgataaaattcatctgttgttgtgatgtctttgaagcctacatatcatcttattgtgcctttcgaaatcttgattagattgacttacattaaaaattggctaattcattcttgaagttatcaatttcaattttttttttcagttgaaatatgaattgcttaatatttaagctagtaattggggaaaaaaaatcaaactggacttccctcccatgtaaagaatgtatttgcagatggttttgaatgtgaaaaatggagattatgagtgtccactgagctgggtgggtataagggcttgggtaggtgggtttcgggcctagagcacatgtgaaggaggtctactggtacaagattgacattttctctttccttaagttcctctggtgattgcaaataacataaattgcctgagcttcttgttttgcgaagaaatcttctgaggtttctcccatgatctctggagttacaaaattattttgctagtatgttccatgctcggttgtccttttcctgtgcaaaaagagttataatactgttcttttgatctgtttttatttgggttaaccaagtatgatgtgatacagaagaatatctgccgccctaccatgtgctgtgagtagtgatccctttgtgttatcctcctattattggactgttttacgaatgactggttctattatgatctctgaggactgatctgttgacaagcaagttttatcaacctccatctgaaaaaaaagaaagtttaatcaacctaaacctaccaatggaagttttagaagttgtatagtttgctggggttggggcctggggaatgagtgtgtacttatttgcttctttatgtaccttccagagagagtaaacaaaggaatagagttatctgttgttggtggatctttctgttgaagtgtgtagttatattggttttgcctgaatatggttgtccatgttttccatccatgtatcttggtaccatcttatttttttctccgtcttacag

SEQ ID NO: 9 - DNA, 129 bp, Solanum melongena
ggagtagtgtactggcaaccacctgcacaagcacttgaaaaggtgaaagaaattatctgggaaccttcagttagtcgctatggtgctgatgagggccttcctgagcttagggaggcgttgatgcaaaag

SEQ ID NO: 10 - DNA, 224 bp, Solanum melongena
gtatggtctatcagctggattactctaatactctggttttcatcgtatgggctgggtagtggaacaaacattggagtggtgtagggtgcttttgccaggtgaaacggtagttactgtcatgtatgaagttggattcatttcatgttttcaaactatatcattcacttgttgagttttggtttttacgttgtttggtctaatactttctttgtgctcttctccag

SEQ ID NO: 11 - DNA, 60 bp, Solanum melongena
ttgggtcatgaaaataacctccataaatcctcggtgatggttactgctggtgctaatcag

SEQ ID NO: 12 - DNA, 1478 bp, Solanum melongena
gtaaaatgttacttttttactattcagtcatctgaggatatagggtcagtcacttcacctctttttcttacctgccctgaatagtagtaggctacctttctttctcgcctttcttccatctttttccagataaaggttggatgttttagaatgaaactgcgttttggagatttgtttgcttgagttagagtgggttgagattgattctaccttcatacaagattcatttgctttgacagaggaccagtatttgggtgcatgtttacttcaccttcctaagctattcttcagttccccttttcccttcattaatgttcaaagttgtctagttcatactagaaacacggcagggctcctcttaaaaaaagaaagtgcaattttctactttttgcattgtcacaatactaagagatttcatctccaaaaccaggaagtgatgcttgtgagggaacgttttccctttctttttacccctctctctatctctctcttaaatgaagatttcttagagtttatgtggtcaagaaaccgtacagtacttttcctgataaatggtatggatacttctgaaagaaaaatagaactgcctcactgataaatggtgtgggattccactaggtatgttgttgttgttgttgttttctctatcatgatgcatacagtatgcagtgtatggaaaggttggtgtgattttgagatttggattttattttcttctgcttctacccatctaaagattattctttttctcgtgtgtatttttcttgataaaaaagatcattcttctgttgtgggcttattcagctccatgttctaacttgatcaaaaaagtcaaatgtgctctctttttcttgtcttttccgttttttgtaataagacctcttttagtttttgcatgttatcactgtacttttgtatgttaccattttcatgagatgacaatcttgcaatgggaacatatgcagcacaaaactctccatttagtatcatctgtcagaaacatatagggaaagaatctactgacatatctagcatgctcaagcacttggccctcacaattttgtctgcaaaatggaacttagggattacttcgactactaatttgagaattaattgcctagattttcaatgactgagtaaatgatggtccaaggggctcagaaagtatgagtacagacacatcattacgtacctgtccattacagagcagtattctctttttgaacaggagaattgtgtcctcaatagtcctccaaattaaaatcacaatttattgcaataaacaaattcggatgaaaccttaagctgaatgaagatagtagagctatgttaatgagccatttgtagagcaatagagttgctacatgtatgggtaaattaattagtgtattgtctatattctttgttagtgactaatggactagctgtatccctatcacttagaaatcactaatggagtctcactgaattgattccag

SEQ ID NO: 13 - DNA, 157 bp, Solanum melongena
gctttcgtaaatgtcgttctcaccctgtgtgatgctggtgattcagttgttatgtttgcaccatactatttcaatgcacacatgtcattccagatgacaggtgttactgatattctggtgggtcctggtgatcccaagacactccatcctgatgcag

SEQ ID NO: 14 - DNA, 634 bp, Solanum melongena
gtttgtaagttcagatgatgttcattttgtgataccctccccattattaagactgctattcctttagtttccttaagactgattacactagatgttgtcatatacatctctgttgtgtagcatgcatgttcaagtttgagggaacatcctttttatctttgtcatctcagcactttggaatatatatcataatcactaatcacatatgtactatgagttacttttttcctctttgcttgaaatttatcaaaaaactccatcttctctgaatctaacactacttgtgcagaaatcaacttaagaagaggttgctgcagaagtagtgttcagctttgtattgcaagttgtgtaaatcattcataatggtctattagtcttgatttgtagaatgttgtctggaaagcaatcattctgtgttttttctcgtattggatgtcctcaccccatccccaccagaaagaaaccaaaaaaaataatgaatttagtaaacttatagtttgacactttgaagcataatgttaacctaaatattgcttctattttgcataatggacttgagagtttcaaaacattatctgccttcgttatttgattgtttatggattgatatattccatgatttctcaattttcag

SEQ ID NO: 15 - DNA, 107 bp, Solanum melongena
actggttggagagtactttaaagaatactgtaccaacaccaaagctcgtcactgttgttaatcctggcaatccatcaggaacatatatccccgagtctcttcttaag

SEQ ID NO: 16 - DNA, 126 bp, Solanum melongena
gtctctatctcatctttatagatatgaatgtattggttgaagtcatcagttattcaaagtgcattactattctcatctgatttttactttattgaaacatcaacaagttgcattttgttcatgtag

SEQ ID NO: 17 - DNA, 59 bp, Solanum melongena
aggatatctgatatttgtaagaaggcaggatgttggctcgtaattgataacacatatga

SEQ ID NO: 18 - DNA, 643 bp, Solanum melongena
gtaagttactttttctgttgcatacgaatcttttagtttctcattttaaattgtgtactggttgttaataactggtgccgatatgttttctcatccatggatgaaagatgacattcttagaactaaagatgatgagggttgttgaatggactaatcctggaatacttttggttagaccagcaagagattattgaataaaccaaggaaacaggtcgtttgcattgcattgtgaggaaatctttttgctttgtgaacctaaacttgaactaaatttgataggcaagaaaatttatggtatcctgggatctgttgccatattttgattgctgagaaggggagaaaggaaatagctaaggtgaaagaatgatcagtctttgaattcatccaaattggcccacttgttgctgtttgttctcaatctctagatggaaaataagcctagaaagttggcttctcaacgagttagatagttaggacacattactattgagtctttcctcctccatgaatgtgaacatcttgttctgtcaaacatcatctctgttccttctttttcttgcaactttttgctttacactctgcttgtcgttttctatattcctgaatgatatgttcttatatatatgttgtaagttatttgcag

SEQ ID NO: 19 - DNA, 109 bp, Solanum melongena
gtatttcatgtatgataatcggaaacatgtttgcatagaagcaaaccacattgtcaacatcttttccttctctaaagcatatgggatgatgggatggagagttggatat

SEQ ID NO: 20 - DNA, 601 bp, Solanum melongena
gtaagtgatgcttgttctaacttatatctagcaatgtaataatattgggcagacaagtgattattattctgctgggtgagcctcaacacaaccagaaaatatacctggttaaaagatgattttttctatgttttccgcaactgcatcttcttgcctcataaactccctcgtctttacctttaaaccaaaaaccaaaaaaaatttaaaaaaattaaactgttgtctttacttatacctctttttaaaaccagcatgtatgacacctttaatcagtctctctatccttgtccatcattaacttttataacgaataatgttgcgtcctgtcatttgtgcctggttgagtgatctgctggaattggatataaaattggcctcaataacaaccaaaatacaagtgttcttttgcaacaaaaaggagttgttccaacagctaagacttatggcatatgagacatgattgctttaccagatgtttttgctgcaatgtaaattttgcagcaaaattcctcagcaaacttttgtactgaagatttactcctgaatggagaaggttgtttcatcttgtgagtgagctaaactcatgtcttaatcgatgcag

SEQ ID NO: 21 - DNA, 696 bp, Solanum melongena
atagcatacccatcggaagtggaagggcttgcagctcaactccttaaagttcaggacaacataccaatctgtgcttcaataatctcacaacgactggctctttactcaatggaaatgggaccagaatgggtaactaatcaagtaaaagaccttgtcaagaacagagaggtgcttctagaagccttatctcctttgggaaagggagctgttaaagggggagaaggtgccatttacctgtgggcaaagctgccagataaatacatggacgacttcaaagtagttcactggctagctaagaggcatggagtagtcctgatccctggaagttccagcggttgtccaggttatgttagggtctcctttggaggattgatcgagaaggactgtcgagcagctgcagaaaggctcagaaaaggtttggaagagctggtaaatagtggaatggcgtcatgattctctctgactaaaatttagtgtcagctggttctcctggacatcagtcatcaacaatacaatgacagacactttctatccttaataattgaagggttttaagctttgcaacttgatcattggacatgcaagttaaaacttgccattctgtatagtttgaaatgaagtattcatagatacctacttttcttaaatggatgatggaagtgtctcatttatctcagagcatatctcattgaatca

SEQ ID NO: 22 - DNA, 2000 bp, Solanum melongena
gaaaataaaaataaatgcgacgtgcctcgaagtttcgcaattcaagaatccccgaaacttcatttgtttcccaaataacgataaataaataaataaatatcctctccatccaattgatcattacttgtttattactctctctgtctcattttaattaaacttgtgagattaatatatacatattaaaaaaaatattcgaagacaaaatttatatcatacttttcactattgcccttcgtaaaatcataaatatatagtgtaacttatctcttagaaaatataaaagtttaataaataaaagggcaaaaataaaaaaaatctcaaacattcatcctgaactttgaacaattcaattattttgaaccttgaaaaaaagttttaaaactttgtaaatatatattactacttatagattgattaataatatatgtttagcctagaaaattaataaattatttatttgttgtttgtatctattctatttttattattatataatactattcaatatttcatatattttctaccacatttgtattaaatatattcaaaggataatattatctttactattatttattgtttaaataaagtgtgtccaaattaaggtgaataactgttgttagacgtagaaattaaataccccacaaggtatccatactgatatcactttttttttaattagatatctattatttgaatgaatatgacaagaatcttctcctttaaaatcaaatttaaattaattgagattttgatatatagtgaattaaatatgaaattaaaaaataaaagtcaatacgagcccttagatcgaagaagtactagggggaggtgattagacatgatatgccgaaatttaatctcattgaggacatgaccctagataggtagacgtagaggtcgcgaattagaatagtaggataattggttggtagggttaggtggttacctagtcagggggcctaacagggttgagtagtaatatttttttttctagcatgagttgtcattatttgttgcttatatgttaattgtattatatttttgtattatcatgtgctttcttttacttttgtcatatctagtcctttctgagtatggattttaaaatgagggttcccagaaacagtctctctacttaggcagtgataaggtctgcatacattctaccctccctagactccacttatgagattttactgattatattgttgttgttgttgatataattttatttattctattcatgtaccaaaagattcctgaagagatcattttataagaaataacaataataatgaaataactttataaatatgagataattttatctttttccaaccaaacaacccataaatttagggaaacatttactccggaaatataataattactccatcaattttaatttatttatcatatatttttttaaaaactatttttatatatttttttcatttcattttatgtgacacacacatatttaaaaaaaacttttaaaattttatggtttaaaatcgctcttaaatatttgtattgctgaaaattatttcattaaaaataaaatataaaaataaactatttctaattttaataagataatatttttctaagacaatgaataaaaatttagaaagccttcattattttcttaaatcctattaaaataggataacagaaactgaggttgtagaacattttaggggttgaatttgatgaattggacagtaggtgggggatagggcaagaaggcagcaaaaagggtgagaaaaacagaaagaaagaaaggcatacagagaatttcccccttttttttctcttaccaaaattaatggacaattcaacttctaacagtcaaacaaattcctaacatatgcagctataacgtggataaagcagaaaaatacaaaaaaaaggtttccatctttttggcatttgcctttgccagctattactatattattaattcccagttgcagttagcagtttcaagggtt

SEQ ID NO: 23 - DNA, 1000 bp, Solanum melongena
ttatacatatgtgtccattggctgatgtatagctaagctaagaagatgccttccagttaagtggatatgctatggtatataacagaaatattaggtctgaatccagttacaacacttagctagttgctgatgaattaatcgagatatgcataagttattcaccaaactcctatagaaaaaatttatgatagaaatatgccattagagtcactttagtaggatatgtgaaagatttttttctcaataaatttctctttcattgttagctagctattgttaaccctcttgggactatagttgatacaatgagctacttagtctttagatttatcaagaggggctcaaacttatattgtggcatatctaggtgtattttcgagtccacgtgaacctacactaggctctcgagattatatatagtagtttacactttttaaaaatacttatatataaatgtgtgaatctacgctcaaaatattatataatatgatgatgattagatgtaacttttcgcaatagtgcactattttttcaaaaattttaatatgcctgaccaagtataaacctagtagatatgaatgattgataattttcacttcatgtttttatgcaaaatggattcataaatacaagcgtactctattaatagtaacaaataaggaccaaatgtgtatcactttccaaagtaaggggtgaaattcaggaataaaacagccagctaggatggagttggattttacattttaaggactttgttaccttataataaccaaaaacattataaattacaataataatttgttctataaaaccgttttagtcaaaccagtcaaaacttcatctgttttttttttccttcttttgtcagaggccattactgccaacccatgataaagaaataccgactttcttttctcatttttaaccttctttcattttcttgaattttgaactttgaactccatcatcccgcctctctcacatttctatctccattttc

SEQ ID NO: 24 - DNA, 9528 bp, Solanum melongena
gaaaataaaaataaatgcgacgtgcctcgaagtttcgcaattcaagaatccccgaaacttcatttgtttcccaaataacgataaataaataaataaatatcctctccatccaattgatcattacttgtttattactctctctgtctcattttaattaaacttgtgagattaatatatacatattaaaaaaaatattcgaagacaaaatttatatcatacttttcactattgcccttcgtaaaatcataaatatatagtgtaacttatctcttagaaaatataaaagtttaataaataaaagggcaaaaataaaaaaaatctcaaacattcatcctgaactttgaacaattcaattattttgaaccttgaaaaaaagttttaaaactttgtaaatatatattactacttatagattgattaataatatatgtttagcctagaaaattaataaattatttatttgttgtttgtatctattctatttttattattatataatactattcaatatttcatatattttctaccacatttgtattaaatatattcaaaggataatattatctttactattatttattgtttaaataaagtgtgtccaaattaaggtgaataactgttgttagacgtagaaattaaataccccacaaggtatccatactgatatcactttttttttaattagatatctattatttgaatgaatatgacaagaatcttctcctttaaaatcaaatttaaattaattgagattttgatatatagtgaattaaatatgaaattaaaaaataaaagtcaatacgagcccttagatcgaagaagtactagggggaggtgattagacatgatatgccgaaatttaatctcattgaggacatgaccctagataggtagacgtagaggtcgcgaattagaatagtaggataattggttggtagggttaggtggttacctagtcagggggcctaacagggttgagtagtaatatttttttttctagcatgagttgtcattatttgttgcttatatgttaattgtattatatttttgtattatcatgtgctttcttttacttttgtcatatctagtcctttctgagtatggattttaaaatgagggttcccagaaacagtctctctacttaggcagtgataaggtctgcatacattctaccctccctagactccacttatgagattttactgattatattgttgttgttgttgatataattttatttattctattcatgtaccaaaagattcctgaagagatcattttataagaaataacaataataatgaaataactttataaatatgagataattttatctttttccaaccaaacaacccataaatttagggaaacatttactccggaaatataataattactccatcaattttaatttatttatcatatatttttttaaaaactatttttatatatttttttcatttcattttatgtgacacacacatatttaaaaaaaacttttaaaattttatggtttaaaatcgctcttaaatatttgtattgctgaaaattatttcattaaaaataaaatataaaaataaactatttctaattttaataagataatatttttctaagacaatgaataaaaatttagaaagccttcattattttcttaaatcctattaaaataggataacagaaactgaggttgtagaacattttaggggttgaatttgatgaattggacagtaggtgggggatagggcaagaaggcagcaaaaagggtgagaaaaacagaaagaaagaaaggcatacagagaatttcccccttttttttctcttaccaaaattaatggacaattcaacttctaacagtcaaacaaattcctaacatatgcagctataacgtggataaagcagaaaaatacaaaaaaaaggtttccatctttttggcatttgcctttgccagctattactatattattaattcccagttgcagttagcagtttcaagggttgtccgtagcagtcaaatttattcatatttaacaaaaagatccaatttttatattttttacaatccctttatataggttccaagctttttgtaagattttcagaaagggaaaggccttttttgctctgtgggtaggtggataagaactcttttcttgaaggtagtgtttattttattgtttttactgagaaagaggaaatgggttctttcggaatgctcgctagaagagctgttcttaccgatacaccagttatggttcaggtaaattacaagatcctagattggatttcttgctcttttgtttggtttaaggttctgtgctttaatgggatatgttgttgttgtgttttgcaatcgatagatacaagaactgattcgaggtaataaagattgtatttctctagctcaggtttgtttactttctccaatgtttgtttcattttgttttactatatcttagttttattattctacttttcattgaatggttcaaaaagttgagaactttgataaaattcatctgttgttgtgatgtctttgaagcctacatatcatcttattgtgcctttcgaaatcttgattagattgacttacattaaaaattggctaattcattcttgaagttatcaatttcaattttttttttcagttgaaatatgaattgcttaatatttaagctagtaattggggaaaaaaaatcaaactggacttccctcccatgtaaagaatgtatttgcagatggttttgaatgtgaaaaatggagattatgagtgtccactgagctgggtgggtataagggcttgggtaggtgggtttcgggcctagagcacatgtgaaggaggtctactggtacaagattgacattttctctttccttaagttcctctggtgattgcaaataacataaattgcctgagcttcttgttttgcgaagaaatcttctgaggtttctcccatgatctctggagttacaaaattattttgctagtatgttccatgctcggttgtccttttcctgtgcaaaaagagttataatactgttcttttgatctgtttttatttgggttaaccaagtatgatgtgatacagaagaatatctgccgccctaccatgtgctgtgagtagtgatccctttgtgttatcctcctattattggactgttttacgaatgactggttctattatgatctctgaggactgatctgttgacaagcaagttttatcaacctccatctgaaaaaaaagaaagtttaatcaacctaaacctaccaatggaagttttagaagttgtatagtttgctggggttggggcctggggaatgagtgtgtacttatttgcttctttatgtaccttccagagagagtaaacaaaggaatagagttatctgttgttggtggatctttctgttgaagtgtgtagttatattggttttgcctgaatatggttgtccatgttttccatccatgtatcttggtaccatcttatttttttctccgtcttacagggagtagtgtactggcaaccacctgcacaagcacttgaaaaggtgaaagaaattatctgggaaccttcagttagtcgctatggtgctgatgagggccttcctgagcttagggaggcgttgatgcaaaaggtatggtctatcagctggattactctaatactctggttttcatcgtatgggctgggtagtggaacaaacattggagtggtgtagggtgcttttgccaggtgaaacggtagttactgtcatgtatgaagttggattcatttcatgttttcaaactatatcattcacttgttgagttttggtttttacgttgtttggtctaatactttctttgtgctcttctccagttgggtcatgaaaataacctccataaatcctcggtgatggttactgctggtgctaatcaggtaaaatgttacttttttactattcagtcatctgaggatatagggtcagtcacttcacctctttttcttacctgccctgaatagtagtaggctacctttctttctcgcctttcttccatctttttccagataaaggttggatgttttagaatgaaactgcgttttggagatttgtttgcttgagttagagtgggttgagattgattctaccttcatacaagattcatttgctttgacagaggaccagtatttgggtgcatgtttacttcaccttcctaagctattcttcagttccccttttcccttcattaatgttcaaagttgtctagttcatactagaaacacggcagggctcctcttaaaaaaagaaagtgcaattttctactttttgcattgtcacaatactaagagatttcatctccaaaaccaggaagtgatgcttgtgagggaacgttttccctttctttttacccctctctctatctctctcttaaatgaagatttcttagagtttatgtggtcaagaaaccgtacagtacttttcctgataaatggtatggatacttctgaaagaaaaatagaactgcctcactgataaatggtgtgggattccactaggtatgttgttgttgttgttgttttctctatcatgatgcatacagtatgcagtgtatggaaaggttggtgtgattttgagatttggattttattttcttctgcttctacccatctaaagattattctttttctcgtgtgtatttttcttgataaaaaagatcattcttctgttgtgggcttattcagctccatgttctaacttgatcaaaaaagtcaaatgtgctctctttttcttgtcttttccgttttttgtaataagacctcttttagtttttgcatgttatcactgtacttttgtatgttaccattttcatgagatgacaatcttgcaatgggaacatatgcagcacaaaactctccatttagtatcatctgtcagaaacatatagggaaagaatctactgacatatctagcatgctcaagcacttggccctcacaattttgtctgcaaaatggaacttagggattacttcgactactaatttgagaattaattgcctagattttcaatgactgagtaaatgatggtccaaggggctcagaaagtatgagtacagacacatcattacgtacctgtccattacagagcagtattctctttttgaacaggagaattgtgtcctcaatagtcctccaaattaaaatcacaatttattgcaataaacaaattcggatgaaaccttaagctgaatgaagatagtagagctatgttaatgagccatttgtagagcaatagagttgctacatgtatgggtaaattaattagtgtattgtctatattctttgttagtgactaatggactagctgtatccctatcacttagaaatcactaatggagtctcactgaattgattccaggctttcgtaaatgtcgttctcaccctgtgtgatgctggtgattcagttgttatgtttgcaccatactatttcaatgcacacatgtcattccagatgacaggtgttactgatattctggtgggtcctggtgatcccaagacactccatcctgatgcaggtttgtaagttcagatgatgttcattttgtgataccctccccattattaagactgctattcctttagtttccttaagactgattacactagatgttgtcatatacatctctgttgtgtagcatgcatgttcaagtttgagggaacatcctttttatctttgtcatctcagcactttggaatatatatcataatcactaatcacatatgtactatgagttacttttttcctctttgcttgaaatttatcaaaaaactccatcttctctgaatctaacactacttgtgcagaaatcaacttaagaagaggttgctgcagaagtagtgttcagctttgtattgcaagttgtgtaaatcattcataatggtctattagtcttgatttgtagaatgttgtctggaaagcaatcattctgtgttttttctcgtattggatgtcctcaccccatccccaccagaaagaaaccaaaaaaaataatgaatttagtaaacttatagtttgacactttgaagcataatgttaacctaaatattgcttctattttgcataatggacttgagagtttcaaaacattatctgccttcgttatttgattgtttatggattgatatattccatgatttctcaattttcagactggttggagagtactttaaagaatactgtaccaacaccaaagctcgtcactgttgttaatcctggcaatccatcaggaacatatatccccgagtctcttcttaaggtctctatctcatctttatagatatgaatgtattggttgaagtcatcagttattcaaagtgcattactattctcatctgatttttactttattgaaacatcaacaagttgcattttgttcatgtagaggatatctgatatttgtaagaaggcaggatgttggctcgtaattgataacacatatgagtaagttactttttctgttgcatacgaatcttttagtttctcattttaaattgtgtactggttgttaataactggtgccgatatgttttctcatccatggatgaaagatgacattcttagaactaaagatgatgagggttgttgaatggactaatcctggaatacttttggttagaccagcaagagattattgaataaaccaaggaaacaggtcgtttgcattgcattgtgaggaaatctttttgctttgtgaacctaaacttgaactaaatttgataggcaagaaaatttatggtatcctgggatctgttgccatattttgattgctgagaaggggagaaaggaaatagctaaggtgaaagaatgatcagtctttgaattcatccaaattggcccacttgttgctgtttgttctcaatctctagatggaaaataagcctagaaagttggcttctcaacgagttagatagttaggacacattactattgagtctttcctcctccatgaatgtgaacatcttgttctgtcaaacatcatctctgttccttctttttcttgcaactttttgctttacactctgcttgtcgttttctatattcctgaatgatatgttcttatatatatgttgtaagttatttgcaggtatttcatgtatgataatcggaaacatgtttgcatagaagcaaaccacattgtcaacatcttttccttctctaaagcatatgggatgatgggatggagagttggatatgtaagtgatgcttgttctaacttatatctagcaatgtaataatattgggcagacaagtgattattattctgctgggtgagcctcaacacaaccagaaaatatacctggttaaaagatgattttttctatgttttccgcaactgcatcttcttgcctcataaactccctcgtctttacctttaaaccaaaaaccaaaaaaaatttaaaaaaattaaactgttgtctttacttatacctctttttaaaaccagcatgtatgacacctttaatcagtctctctatccttgtccatcattaacttttataacgaataatgttgcgtcctgtcatttgtgcctggttgagtgatctgctggaattggatataaaattggcctcaataacaaccaaaatacaagtgttcttttgcaacaaaaaggagttgttccaacagctaagacttatggcatatgagacatgattgctttaccagatgtttttgctgcaatgtaaattttgcagcaaaattcctcagcaaacttttgtactgaagatttactcctgaatggagaaggttgtttcatcttgtgagtgagctaaactcatgtcttaatcgatgcagatagcatacccatcggaagtggaagggcttgcagctcaactccttaaagttcaggacaacataccaatctgtgcttcaataatctcacaacgactggctctttactcaatggaaatgggaccagaatgggtaactaatcaagtaaaagaccttgtcaagaacagagaggtgcttctagaagccttatctcctttgggaaagggagctgttaaagggggagaaggtgccatttacctgtgggcaaagctgccagataaatacatggacgacttcaaagtagttcactggctagctaagaggcatggagtagtcctgatccctggaagttccagcggttgtccaggttatgttagggtctcctttggaggattgatcgagaaggactgtcgagcagctgcagaaaggctcagaaaaggtttggaagagctggtaaatagtggaatggcgtcatgattctctctgactaaaatttagtgtcagctggttctcctggacatcagtcatcaacaatacaatgacagacactttctatccttaataattgaagggttttaagctttgcaacttgatcattggacatgcaagttaaaacttgccattctgtatagtttgaaatgaagtattcatagatacctacttttcttaaatggatgatggaagtgtctcatttatctcagagcatatctcattgaatcattatacatatgtgtccattggctgatgtatagctaagctaagaagatgccttccagttaagtggatatgctatggtatataacagaaatattaggtctgaatccagttacaacacttagctagttgctgatgaattaatcgagatatgcataagttattcaccaaactcctatagaaaaaatttatgatagaaatatgccattagagtcactttagtaggatatgtgaaagatttttttctcaataaatttctctttcattgttagctagctattgttaaccctcttgggactatagttgatacaatgagctacttagtctttagatttatcaagaggggctcaaacttatattgtggcatatctaggtgtattttcgagtccacgtgaacctacactaggctctcgagattatatatagtagtttacactttttaaaaatacttatatataaatgtgtgaatctacgctcaaaatattatataatatgatgatgattagatgtaacttttcgcaatagtgcactattttttcaaaaattttaatatgcctgaccaagtataaacctagtagatatgaatgattgataattttcacttcatgtttttatgcaaaatggattcataaatacaagcgtactctattaatagtaacaaataaggaccaaatgtgtatcactttccaaagtaaggggtgaaattcaggaataaaacagccagctaggatggagttggattttacattttaaggactttgttaccttataataaccaaaaacattataaattacaataataatttgttctataaaaccgttttagtcaaaccagtcaaaacttcatctgttttttttttccttcttttgtcagaggccattactgccaacccatgataaagaaataccgactttcttttctcatttttaaccttctttcattttcttgaattttgaactttgaactccatcatcccgcctctctcacatttctatctccattttc

SEQ ID NO: 25 - DNA, 4558 bp, Solanum melongena
gtcagtcacttcacctctttttcttacctgccctgaatagtagtaggctacctttctttctcgcctttcttccatctttttccagataaaggttggatgttttagaatgaaactgcgttttggagatttgtttgcttgagttagagtgggttgagattgattctaccttcatacaagattcatttgctttgacagaggaccagtatttgggtgcatgtttacttcaccttcctaagctattcttcagttccccttttcccttcattaatgttcaaagttgtctagttcatactagaaacacggcagggctcctcttaaaaaaagaaagtgcaattttctactttttgcattgtcacaatactaagagatttcatctccaaaaccaggaagtgatgcttgtgagggaacgttttccctttctttttacccctctctctatctctctcttaaatgaagatttcttagagtttatgtggtcaagaaaccgtacagtacttttcctgataaatggtatggatacttctgaaagaaaaatagaactgcctcactgataaatggtgtgggattccactaggtatgttgttgttgttgttgttttctctatcatgatgcatacagtatgcagtgtatggaaaggttggtgtgattttgagatttggattttattttcttctgcttctacccatctaaagattattctttttctcgtgtgtatttttcttgataaaaaagatcattcttctgttgtgggcttattcagctccatgttctaacttgatcaaaaaagtcaaatgtgctctctttttcttgtcttttccgttttttgtaataagacctcttttagtttttgcatgttatcactgtacttttgtatgttaccattttcatgagatgacaatcttgcaatgggaacatatgcagcacaaaactctccatttagtatcatctgtcagaaacatatagggaaagaatctactgacatatctagcatgctcaagcacttggccctcacaattttgtctgcaaaatggaacttagggattacttcgactactaatttgagaattaattgcctagattttcaatgactgagtaaatgatggtccaaggggctcagaaagtatgagtacagacacatcattacgtacctgtccattacagagcagtattctctttttgaacaggagaattgtgtcctcaatagtcctccaaattaaaatcacaatttattgcaataaacaaattcggatgaaaccttaagctgaatgaagatagtagagctatgttaatgagccatttgtagagcaatagagttgctacatgtatgggtaaattaattagtgtattgtctatattctttgttagtgactaatggactagctgtatccctatcacttagaaatcactaatggagtctcactgaattgattccaggctttcgtaaatgtcgttctcaccctgtgtgatgctggtgattcagttgttatgtttgcaccatactatttcaatgcacacatgtcattccagatgacaggtgttactgatattctggtgggtcctggtgatcccaagacactccatcctgatgcaggtttgtaagttcagatgatgttcattttgtgataccctccccattattaagactgctattcctttagtttccttaagactgattacactagatgttgtcatatacatctctgttgtgtagcatgcatgttcaagtttgagggaacatcctttttatctttgtcatctcagcactttggaatatatatcataatcactaatcacatatgtactatgagttacttttttcctctttgcttgaaatttatcaaaaaactccatcttctctgaatctaacactacttgtgcagaaatcaacttaagaagaggttgctgcagaagtagtgttcagctttgtattgcaagttgtgtaaatcattcataatggtctattagtcttgatttgtagaatgttgtctggaaagcaatcattctgtgttttttctcgtattggatgtcctcaccccatccccaccagaaagaaaccaaaaaaaataatgaatttagtaaacttatagtttgacactttgaagcataatgttaacctaaatattgcttctattttgcataatggacttgagagtttcaaaacattatctgccttcgttatttgattgtttatggattgatatattccatgatttctcaattttcagactggttggagagtactttaaagaatactgtaccaacaccaaagctcgtcactgttgttaatcctggcaatccatcaggaacatatatccccgagtctcttcttaaggtctctatctcatctttatagatatgaatgtattggttgaagtcatcagttattcaaagtgcattactattctcatctgatttttactttattgaaacatcaacaagttgcattttgttcatgtagaggatatctgatatttgtaagaaggcaggatgttggctcgtaattgataacacatatgagtaagttactttttctgttgcatacgaatcttttagtttctcattttaaattgtgtactggttgttaataactggtgccgatatgttttctcatccatggatgaaagatgacattcttagaactaaagatgatgagggttgttgaatggactaatcctggaatacttttggttagaccagcaagagattattgaataaaccaaggaaacaggtcgtttgcattgcattgtgaggaaatctttttgctttgtgaacctaaacttgaactaaatttgataggcaagaaaatttatggtatcctgggatctgttgccatattttgattgctgagaaggggagaaaggaaatagctaaggtgaaagaatgatcagtctttgaattcatccaaattggcccacttgttgctgtttgttctcaatctctagatggaaaataagcctagaaagttggcttctcaacgagttagatagttaggacacattactattgagtctttcctcctccatgaatgtgaacatcttgttctgtcaaacatcatctctgttccttctttttcttgcaactttttgctttacactctgcttgtcgttttctatattcctgaatgatatgttcttatatatatgttgtaagttatttgcaggtatttcatgtatgataatcggaaacatgtttgcatagaagcaaaccacattgtcaacatcttttccttctctaaagcatatgggatgatgggatggagagttggatatgtaagtgatgcttgttctaacttatatctagcaatgtaataatattgggcagacaagtgattattattctgctgggtgagcctcaacacaaccagaaaatatacctggttaaaagatgattttttctatgttttccgcaactgcatcttcttgcctcataaactccctcgtctttacctttaaaccaaaaaccaaaaaaaatttaaaaaaattaaactgttgtctttacttatacctctttttaaaaccagcatgtatgacacctttaatcagtctctctatccttgtccatcattaacttttataacgaataatgttgcgtcctgtcatttgtgcctggttgagtgatctgctggaattggatataaaattggcctcaataacaaccaaaatacaagtgttcttttgcaacaaaaaggagttgttccaacagctaagacttatggcatatgagacatgattgctttaccagatgtttttgctgcaatgtaaattttgcagcaaaattcctcagcaaacttttgtactgaagatttactcctgaatggagaaggttgtttcatcttgtgagtgagctaaactcatgtcttaatcgatgcagatagcatacccatcggaagtggaagggcttgcagctcaactccttaaagttcaggacaacataccaatctgtgcttcaataatctcacaacgactggctctttactcaatggaaatgggaccagaatgggtaactaatcaagtaaaagaccttgtcaagaacagagaggtgcttctagaagccttatctcctttgggaaagggagctgttaaagggggagaaggtgccatttacctgtgggcaaagctgccagataaatacatggacgacttcaaagtagttcactggctagctaagaggcatggagtagtcctgatccctggaagttccagcggttgtccaggttatgttagggtctcctttggaggattgatcgagaaggactgtcgagcagctgcagaaaggctcagaaaaggtttggaagagctggtaaatagtggaatggcgtcatgattctctctgactaaaatttagtgtcagctggttctcctggacatcagtcatcaacaatacaatgacagacactttctatccttaataattgaagggttttaagctttgcaacttgatcattggacatgcaagttaaaacttgccattctgtatagtttgaaatgaagtattcatagatacctacttttcttaaatggatgatggaagtgtctcatttatctcagagcatatctca

SEQ ID NO: 26 - DNA, 227 bp, Solanum melongena
tatggtatataacagaaatattaggtctgaatccagttacaacacttagctagttgctgatgaattaatcgagatatgcataagttattcaccaaactcctatagaaaaaatttatgatagaaatatgccattagagtcactttagtaggatatgtgaaagatttttttctcaataaatttctctttcattgttagctagctattgttaaccctcttgggactatag

SEQ ID NO: 27 - DNA, 1339 bp, Solanum melongena
ttgggtcatgaaaataacctccataaatcctcggtgatggttactgctggtgctaatcaggtaaaatgttacttttttactattcagtcatctgaggatataggtatggtatataacagaaatattaggtctgaatccagttacaacacttagctagttgctgatgaattaatcgagatatgcataagttattcaccaaactcctatagaaaaaatttatgatagaaatatgccattagagtcactttagtaggatatgtgaaagatttttttctcaataaatttctctttcattgttagctagctattgttaaccctcttgggactatagttgaatcattatacatatgtgtccattggctgatgtatagctaagctaagaagatgccttccagttaagtggatatgctatggtatataacagaaatattaggtctgaatccagttacaacacttagctagttgctgatgaattaatcgagatatgcataagttattcaccaaactcctatagaaaaaatttatgatagaaatatgccattagagtcactttagtaggatatgtgaaagatttttttctcaataaatttctctttcattgttagctagctattgttaaccctcttgggactatagttgatacaatgagctacttagtctttagatttatcaagaggggctcaaacttatattgtggcatatctaggtgtattttcgagtccacgtgaacctacactaggctctcgagattatatatagtagtttacactttttaaaaatacttatatataaatgtgtgaatctacgctcaaaatattatataatatgatgatgattagatgtaacttttcgcaatagtgcactattttttcaaaaattttaatatgcctgaccaagtataaacctagtagatatgaatgattgataattttcacttcatgtttttatgcaaaatggattcataaatacaagcgtactctattaatagtaacaaataaggaccaaatgtgtatcactttccaaagtaaggggtgaaattcaggaataaaacagccagctaggatggagttggattttacattttaaggactttgttaccttataataaccaaaaacattataaattacaataataatttgttctataaaaccgttttagtcaaaccagtcaaaacttcatctgttttttttttccttcttttgtcagaggccattactgccaacccatgataaagaaataccgactttcttttctcatttttaaccttctttcattttcttgaattttgaactttgaactccatcatcccgcctctctcacatttctatctccattttc

SEQ ID NO: 28 - protein, 394 aa, Solanum lycopersicum
MGSFGMLARRAVLTETPVMVQIQELVRSNKGCISLAQGVVYWQPPAQALEKVKEAIWEPSVSRYGADEGLPELREALMQKLGRENNLHKSSVMVTAGANQAFVNVVLTLCDAGDSVVMFAPYYFNAHMSFQMTGVTDILVGPGDAKTLHPDADWLESTLKNTVPTPKLVTVVNPGNPSGTYIPESLLKRISDICKEAGCWLVIDNTYEYFMYDDRKHVCIEANHIVNIFSFSKAYGMMGWRVGYIAYPSEVEGLAVQLLKVQDNIPICASIISQRLALYSMEMGPEWVANQVKDLVKNREVLQEALSPLGEGAVKGGEAAIYLWAKLPDKYMDDFKVVHWLAKRHGVVLIPGSSSGCPGYLRIAFGGLIEKDCRVAAERLRKGLEELVNFGMVS

SEQ ID NO: 29 - DNA, 1185 bp, Solanum lycopersicum
atggggtcttttggaatgcttgctagaagggctgtgcttaccgagacaccagttatggttcagatacaagaactggttcgaagtaataaaggttgtatttctctagctcagggagtagtgtactggcaaccacctgcgcaagcacttgaaaaggtgaaagaagctatctgggaaccttcagttagtcgctatggtgccgatgagggccttcctgaacttagggaggcattgatgcaaaagttgggtcgtgaaaataacctacataaatcttcagtgatggttactgccggtgcaaatcaggctttcgtaaatgtcgttctcacactgtgtgatgctggggattcggtcgttatgtttgcaccatactatttcaatgcacacatgtcattccagatgacaggtgttaccgatattctggtgggtcctggtgatgcaaagacactccatcctgatgcagactggttggagagtactctaaagaatactgtaccaaccccaaagcttgtcactgttgttaatcccggcaatccatcaggaacatatattcctgagtcccttcttaagaggatatctgatatttgtaaggaagcgggatgttggctcgtaattgataacacatatgagtattttatgtatgatgatcgcaagcatgtttgcatagaagcaaaccacattgtcaacatcttttccttctccaaagcatatgggatgatgggatggcgagttggatatatagcatacccatcggaagtggaagggcttgcagttcaactccttaaagttcaggacaacataccgatttgtgcttcaataatctcacaacgactggctctctactcaatggaaatgggaccagaatgggtagctaatcaagttaaggaccttgtcaagaacagagaggtgctacaagaagccttatctcctttgggagagggggctgttaaagggggagaagctgccatttacctgtgggcaaagctgccagataaatacatggacgacttcaaagtagttcactggctagctaagaggcatggagtagtcctgatccctggaagttccagcggttgtccaggttatcttaggatcgcctttggaggattgattgagaaggactgtcgagtagctgcagaaaggctcagaaaaggtttggaagagctggtaaattttggaatggtttcatga

SEQ ID NO: 30 - protein, 394 aa, Solanum pimpinellifolium; identical to SEQ ID NO: 28

SEQ ID NO: 31 - DNA, 1185 bp, Solanum pimpinellifolium
atggggtcttttggaatgcttgctagaagggctgtgcttaccgagacaccagttatggttcagatacaagaactggttcgaagtaataaaggttgtatttctctagctcagggagtagtgtactggcaaccacctgcgcaagcacttgaaaaggtgaaagaagctatctgggaaccttcagttagtcgctatggtgccgatgagggccttcctgaacttagggaggcgttgatgcaaaagttgggtcgtgaaaataacctacataaatcttcagtgatggttactgccggtgcaaatcaggctttcgtaaatgtcgttctcacactgtgtgatgctggggattcggtcgttatgtttgcaccatactatttcaatgcacacatgtcattccagatgacaggtgttaccgatattctggtgggtcctggtgatgcaaagacactccatcctgatgcagactggttggagagtactctaaagaatactgtaccaaccccaaagcttgtcactgttgttaatcccggcaatccatcaggaacatatattcctgagtcccttcttaagaggatatctgatatttgtaaggaagcgggatgttggctcgtaattgataacacatatgagtattttatgtatgatgatcgcaagcatgtttgcatagaagcaaaccacattgtcaacatcttttccttctccaaagcatatgggatgatgggatggcgagttggatatatagcatacccatcggaagtggaagggcttgcagttcaactccttaaagttcaggacaacataccgatttgtgcttcaataatctctcaacgactggctctctactcaatggaaatgggaccagaatgggtagctaatcaagttaaggaccttgtcaagaacagagaggtgctacaagaagccttatctcctttgggagagggggctgttaaagggggagaagctgccatttacctgtgggcaaagctgccagataaatacatggacgacttcaaagtagttcactggctagctaagaggcatggagtagtcctgatccctggaagttccagcggttgtccaggttatcttaggatcgcctttggaggattgattgagaaggactgtcgagtagctgcagaaaggctcagaaaaggtttggaagagctggtaaattttggaatggtttcatga

SEQ ID NO: 32 - protein, 394 aa, Solanum tuberosum phureja
MGSFGMLARRAVLTETPVMVQIQELVRGNKDCISLAQGVVYWQPPARALEKVKEAIWEPSVSRYGADEGLPELREALIQKLGRENNLHKSSVMVTAGANQAFVNVVLTLCDAGDSVVMFAPYYFNAHMSFQMTGVTDILVGPGDAKTLHPDADWLESTLKNTVPTPKLVTVVNPGNPSGTYIPESLLKRISDICKEAGCWLVIDNTYEYFMYDDRKHVCIEANHIVNIFSFSKAYGMMGWRVGYIAYPSEVEGLAAQLLKVQDNIPICASIISQRLALYSMEMGPEWVTNQVKDLVKNREVLQEALSPLGEEAVKGGEGAIYLWAKLPDKYMDDFKVVHWLAKRHGIVLIPGSSSGCPGYVRIAFGGLIEKDCRVAAERLRKGLEELVNSGMVS

SEQ ID NO: 33 - DNA, 1185 bp, Solanum tuberosum phureja
atggggtcttttggaatgcttgctagaagagctgtgcttaccgagacaccagttatggttcagatacaagaactggttcgaggtaataaagattgtatttctctagctcagggagtagtgtactggcaaccacctgcgcgagcacttgaaaaggtgaaagaagctatctgggaaccttcagttagtcgctatggtgccgatgagggccttcctgagcttagggaggcgttgattcaaaagttgggtcgtgaaaataacctacataaatcctcagtgatggttactgctggtgcaaatcaggctttcgtaaatgtcgttctcacactgtgtgatgctggcgattcggtcgttatgtttgcaccatactatttcaatgcacacatgtcattccagatgacaggtgttaccgatattctggtgggtcctggtgatgcaaagacactccatcctgatgcagactggttggagagtactctaaagaatactgtaccaaccccaaagcttgtcactgttgttaatcccggcaatccatcaggaacgtatatccctgagtcccttcttaagaggatatctgatatttgtaaggaagcgggatgttggctcgtaattgataacacatatgagtatttcatgtatgatgatcggaagcatgtttgcatagaagcaaaccacattgtcaacatcttttccttctccaaagcatatgggatgatgggatggcgagttggatatatagcatacccatcggaagtggaagggctcgcagctcaactccttaaagttcaggacaacataccgatttgtgcttcaataatctcacaacgactggctctttactccatggaaatgggaccagaatgggtaactaatcaagttaaagaccttgtcaagaacagagaggtgcttcaagaagccttatctcctttgggagaggaagctgttaaagggggagaaggtgccatttacctgtgggcaaagctgccagataaatacatggacgacttcaaagtagttcactggttagctaagaggcatggaatagttctgatccctggaagttccagcggttgtccaggttatgttaggatcgcctttggaggattgattgagaaggactgtcgagtagctgcagaaaggctcagaaaaggtttggaagagctggtaaatagtggaatggtttcatga

SEQ ID NO: 34 - protein, 394 aa, Capsicum annuum
MGSFGMLARRAVLTETPVMVQIQELVRGLKDCVSLAQGVVYWQPPAQALEKVKEIIWEPSVSRYGADEGLPELREALKQKLGRENNLHKSSVMVTSGANQAFVNVVLALCDAGDSVVMFAPYYFNAYMSFQMTGVTDILVGSVDAKTLQPDADWLESTLKNTVPTPKLVTVVNPGNPSGTYIPESLLKRISDICKEAGCWLVVDNTYEYFMYDDRKHVCVEANHIVNIFSFSKAYGMMGWRVGYIAYPSEVDGLAAQLLKVQDNIPICASIISQRLALYSMEVGPEWVADQVKNLVKNRDVLLEALSPLGEEAVKGGEGALYLWVKLPDKYADDVKVVHWLAKRHGVVLIPGSSCGCPGFVRISFGGLIEKDTITAAKRLRKGLEELLDSGMDS

SEQ ID NO: 35 - DNA, 1185 bp, Capsicum annuum
atgggttcttttggaatgctagctagaagagctgttcttacagaaacacctgttatggttcagattcaagaattggtacgaggtcttaaagattgtgtttctttagctcagggagtagtgtactggcaaccacctgcgcaagcacttgaaaaggtgaaagaaattatctgggaaccttcagttagtcgctatggtgccgatgagggccttcctgagctcagggaggcgttgaaacaaaagttgggtcgtgaaaataacctacataaatcctcagtgatggttacttctggtgcaaatcaggcttttgtaaatgtcgttctcgcactgtgtgatgctggtgattcggttgtcatgtttgcaccatactatttcaatgcatacatgtcattccagatgacgggtgttaccgatattctggtgggttctgttgatgcaaagacactccagcctgatgcagactggttggagagtactctaaagaatactgtaccaaccccaaagcttgtcactgttgttaatcccggcaatccgtcaggaacatatatccctgagtcccttcttaagaggatatctgatatttgtaaggaagcgggatgttggctcgtagttgataacacatatgagtatttcatgtatgatgataggaagcatgtttgcgtagaagcaaaccacattgtaaacatcttttccttctctaaagcatatgggatgatgggatggagagttggatatatagcatacccatcggaagtggacgggctcgcagctcaactccttaaagttcaggacaacatacctatttgtgcttcgataatctcacaacgactggctctttactcaatggaagtgggaccagaatgggtagctgatcaagtaaaaaacctcgtcaagaacagagatgtacttctagaagctctctctcctttgggagaggaagctgttaaagggggagaaggtgccctttacctgtgggtaaagctgcccgataagtacgcggacgacgttaaagtagttcactggctagctaagaggcatggagtagtcctgatccccggcagttcctgcggctgtccaggttttgttagaatctccttcggaggattgattgaaaaggacactataacagctgcaaaaaggctcagaaaaggtttggaagagctgttagatagtggaatggattcatga

SEQ ID NO: 36 - protein, 394 aa, Malus domestica
MGSYGQLARRAVETNMPIMVQIQQLVRGAKNAVSLAQGVVYWQPPKQALDKVRELVWEPSISRYGADEGIPELREALVQKLHRENKLYKSSVMVTAGANQAFVNLALTLCDAGDSVVMFAPYYFNAYMSFQMTGVTNILVGPGHPKTLYPDADWLEKTLSETKPTPKLVTVVNPGNPSGTYIPDSLLKRISDICRDAGSWLVVDNTYEYFMYDDLKHTCVEGNHIINIFSFSKAYGMMGWRVGYIAYPSEVEGFGTQLLKVQDNIPICASIISQHLALHSLEMGPEWVTERVKGLVKNREIVLEALSPLGDNAVKGGEGAIYLWAKLPDKYVDDDKFVHWLAHRHGVVVIPGSACGCPGNVRISFGGLVEDDCKAAAERLRRGFEELIRDGMVE

SEQ ID NO: 37 - DNA, 1185 bp, Malus domestica
atgggttcctatggacaacttgcaaggagggctgtggagactaatatgccgatcatggttcagatacagcagctggtccgaggagccaaaaatgccgtgtcactggctcagggagtggtttattggcaaccacccaagcaggcattggacaaggtgagagaacttgtttgggagccttcaattagtcgttacggtgctgatgaaggtatacctgaactcagggaggcattggtacaaaagttgcatcgtgaaaataagttgtacaaatcttcagtgatggttactgcaggcgcaaatcaggcatttgtgaaccttgctcttacattgtgtgatgccggagactctgtggtaatgtttgcaccatactacttcaatgcttacatgtcctttcagatgacaggagtcactaatatactcgtgggtcctggtcacccaaagacactctacccagatgcagactggttggagaaaacgttatccgaaaccaaaccaaccccaaaacttgttacagttgttaatcctggcaacccaagtggaacctatattccggattctcttcttaagaggatatctgatatatgcagagatgctggatcctggctagttgtggataatacatatgagtattttatgtatgatgatttgaaacacacatgtgtggagggaaatcacataatcaacattttttccttctcgaaagcttatgggatgatgggatggcgtgttggatatatagcttacccatcagaagtagagggctttggtacccaactcctcaaagttcaggataacattcccatctgtgcttcaataatttcgcagcaccttgccctccactcattggaaatgggacccgaatgggtcactgaacgagtgaaaggtctagtcaagaacagagaaattgttctagaagctctctctcccctcggggacaatgctgttaaaggtggagaaggtgctatatacttgtgggcaaagcttccggacaaatatgtagatgatgataaatttgttcactggcttgctcacaggcatggggtggtggtgatccccggaagtgcttgtggatgcccggggaatgtgagaatctccttcggtggcttggtggaggatgactgcaaagctgctgcagaaaggctgaggagagggttcgaagagttgatcagagatggaatggtcgagtaa

SEQ ID NO: 38 - protein, 355 aa, Solanum melongena
MGSFGMLARRAVLTDTPVMVQIQELIRGNKDCISLAQGVVYWQPPAQALEKVKEIIWEPSVSRYGADEGLPELREALMQKLGHENNLHKSSVMVTAGANQVNEGVQLKVNCLGNYMPLHTYYEERKFSNLSFNAYGSNYKISSYCPKIHGCMHCTTAKAAGSETRSADRFQHGNPQGEEQESSTYFLCGEEMPASAGCHKSMLQHFKWRLPRYQSPKEEEDHSSWKQLNKCVSDHFSRLSVSISSQVTTKEPSQLLRQEVPTTRKDKRNQRFSKKRHSESYLCGTININKVGRHRHFSKGSTTMQSICLYIEFTGCGANKAAIKFHGNAPARYHTKYAGNPCRLDCGGKLVFIPN

SEQ ID NO: 39 - DNA, 27 bp, Artificial Sequence
  Antisense nucleotide
gccctcatcagcaccatagcgactaac

SEQ ID NO: 40 - DNA, 28 bp, Artificial Sequence
  Antisense nucleotide
gcaccatagcgactaactgaaggttccc

SEQ ID NO: 41 - DNA, 26 bp, Artificial Sequence
  Sense nucleotide
ctgggaaccttcagttagtcgctatg

SEQ ID NO: 42 - DNA, 26 bp, Artificial Sequence
  Sense nucleotide
ttagtcgctatggtgctgatgagggc

SEQ ID NO: 43 - DNA, 30 bp, Artificial Sequence
  Sense nucleotide
ctccccgggtttttgctctgtgggtaggtg

SEQ ID NO: 44 - DNA, 26 bp, Artificial Sequence
  Antisense nucleotide
ctcgagctccaggagaaccagctgac

SEQ ID NO: 45 - DNA, 24 bp, Artificial Sequence
  Sense nucleotide
aagagctgttcttaccgatacacc

SEQ ID NO: 46 - DNA, 23 bp, Artificial Sequence
  Antisense nucleotide
gattagcaccagcagtaaccatc

SEQ ID NO: 47 - DNA, 20 bp, Artificial Sequence
  Sense nucleotide
caaccccatctctcactcgt

SEQ ID NO: 48 - DNA, 20 bp, Artificial Sequence
  Antisense nucleotide
aacaatgtgacagcccacaa

SEQ ID NO: 49 - DNA, 24 bp, Artificial Sequence
  Sense nucleotide
tcatctgaggatatagggtcagtc

SEQ ID NO: 50 - DNA, 23 bp, Artificial Sequence
  Antisense nucleotide
ccaaatctcaaaatcacaccaac

SEQ ID NO: 51 - DNA, 24 bp, Artificial Sequence
  Sense nucleotide
agtcatctgaggatataggtatgg

SEQ ID NO: 52 - DNA, 29 bp, Artificial Sequence
  Antisense nucleotide
ggtaacaaagtccttaaaatgtaaaatcc

SEQ ID NO: 53 - DNA, 22 bp, Artificial Sequence
  Sense nucleotide
tcatttgtttcccaaataacga

SEQ ID NO: 54 - DNA, 29 bp, Artificial Sequence
  Antisense nucleotide
ctccccgggctagcgagcattccgaaaga

SEQ ID NO: 55 - DNA, 2173 bp, Solanum melongena
tcatttgtttcccaaataacgataaataaataaataaatatcctctccatccaattgatcattacttgtttattactctctctgtctcattttaattaaacttgtgagattaatatatacatattaaaaaaaatattcgaagacaaaatttatatcatacttttcactattgcccttcgtaaaatcataaatatatagtgtaacttatctcttagaaaatataaaagtttaataaataaaagggcaaaaataaaaaaaatctcaaacattcatcctgaactttgaacaattcaattattttgaaccttgaaaaaaagttttaaaactttgtaaatatatattactacttatagattgattaataatatatgtttagcctagaaaattaataaattatttatttgttgtttgtatctattctatttttattattatataatactattcaatatttcatatattttctaccacatttgtattaaatatattcaaaggataatattatctttactattatttattgtttaaataaagtgtgtccaaattaaggtgaataactgttgttagacgtagaaattaaataccccacaaggtatccatactgatatcactttttttttaattagatatctattatttgaatgaatatgacaagaatcttctcctttaaaatcaaatttaaattaattgagattttgatatatagtgaattaaatatgaaattaaaaaataaaagtcaatacgagcccttagatcgaagaagtactagggggaggtgattagacatgatatgccgaaatttaatctcattgaggacatgaccctagataggtagacgtagaggtcgcgaattagaatagtaggataattggttggtagggttaggtggttacctagtcagggggcctaacagggttgagtagtaatatttttttttctagcatgagttgtcattatttgttgcttatatgttaattgtattatatttttgtattatcatgtgctttcttttacttttgtcatatctagtcctttctgagtatggattttaaaatgagggttcccagaaacagtctctctacttaggcagtgataaggtctgcatacattctaccctccctagactccacttatgagattttactgattatattgttgttgttgttgatataattttatttattctattcatgtaccaaaagattcctgaagagatcattttataagaaataacaataataatgaaataactttataaatatgagataattttatctttttccaaccaaacaacccataaatttagggaaacatttactccggaaatataataattactccatcaattttaatttatttatcatatatttttttaaaaactatttttatatatttttttcatttcattttatgtgacacacacatatttaaaaaaaacttttaaaattttatggtttaaaatcgctcttaaatatttgtattgctgaaaattatttcattaaaaataaaatataaaaataaactatttctaattttaataagataatatttttctaagacaatgaataaaaatttagaaagccttcattattttcttaaatcctattaaaataggataacagaaactgaggttgtagaacattttaggggttgaatttgatgaattggacagtaggtgggggatagggcaagaaggcagcaaaaagggtgagaaaaacagaaagaaagaaaggcatacagagaatttcccccttttttttctcttaccaaaattaatggacaattcaacttctaacagtcaaacaaattcctaacatatgcagctataacgtggataaagcagaaaaatacaaaaaaaaggtttccatctttttggcatttgcctttgccagctattactatattattaattcccagttgcagttagcagtttcaagggttgtccgtagcagtcaaatttattcatatttaacaaaaagatccaatttttatattttttacaatccctttatataggttccaagctttttgtaagattttcagaaagggaaaggccttttttgctctgtgggtaggtggataagaactcttttcttgaaggtagtgtttattttattgtttttactgagaaagaggaaatgggttctttcggaatgctcgctagcccggggag

SEQ ID NO: 56 - DNA, 35 bp, Artificial Sequence
  Sense nucleotide
ctccccgggaagcttgcaggatgttggctcgtaat

SEQ ID NO: 57 - DNA, 32 bp, Artificial Sequence
  Antisense nucleotide
ctcctcgagctcaacataacctggacaaccgc

SEQ ID NO: 58 - DNA, 522 bp, Artificial Sequence
  PCR product
ctccccgggaagcttgcaggatgttggctcgtaattgataacacatatgagtatttcatgtatgataatcggaaacatgtttgcatagaagcaaaccacattgtcaacatcttttccttctctaaagcatatgggatgatgggatggagagttggatatatagcatacccatcggaagtggaagggcttgcagctcaactccttaaagttcaggacaacataccaatctgtgcttcaataatctcacaacgactggctctttactcaatggaaatgggaccagaatgggtaactaatcaagtaaaagaccttgtcaagaacagagaggtgcttctagaagccttatctcctttgggaaagggagctgttaaagggggagaaggtgccatttacctgtgggcaaagctgccagataaatacatggacgacttcaaagtagttcactggctagctaagaggcatggagtagtcctgatccctggaagttccagcggttgtccaggttatgttgagctcgaggag

SEQ ID NO: 59 - DNA, 35 bp, Artificial Sequence
  Sense nucleotide
ctccccgggatcgatggaggcattgatgcaaaagt

SEQ ID NO: 60 - DNA, 32 bp, Artificial Sequence
  Antisense nucleotide
ctcctcgagctctcccatcatcccatatgctt

SEQ ID NO: 61 - DNA, 523 bp, Artificial Sequence
  PCR product
ctccccgggatcgatggaggcattgatgcaaaagttgggtcgtgaaaataacctacataaatcttcagtgatggttactgccggtgcaaatcaggctttcgtaaatgtcgttctcacactgtgtgatgctggggattcggtcgttatgtttgcaccatactatttcaatgcacacatgtcattccagatgacaggtgttaccgatattctggtgggtcctggtgatgcaaagacactccatcctgatgcagactggttggagagtactctaaagaatactgtaccaaccccaaagcttgtcactgttgttaatcccggcaatccatcaggaacatatattcctgagtcccttcttaagaggatatctgatatttgtaaggaagcgggatgttggctcgtaattgataacacatatgagtattttatgtatgatgatcgcaagcatgtttgcatagaagcaaaccacattgtcaacatcttttccttctccaaagcatatgggatgatgggagagctcgaggag

SEQ ID NO: 62 - DNA, 1908 bp, Solanum lycopersicum
tctgttcctcattaatattctgattttattaatcaagattgtgagtaccaatttgttactcattgattttcctctcctaagatttattcatgattcgatggccgttaatggtgtatttttcaactaggatgatttagatttgacttctatatgaatatttcatgacttttatgaaatatttcgagatcgtgatttttctatgaaatttttgagatgtcttttaagagaatttagcagtctttatatagacagaaactaggatttatgattgagtagcttccgaaaattctaataaaatcccaacttgaatcgaacatattttgttaaatcctacgaaatttcaccgtatacagatctctttaaaaaaatccattcctataagggaagaacaaatatataacgattctattcgtataaggaataagttcctatacttattagaggagtggataagcttctcagtatcaacatgcatgtttgatgtctcttcaaatatggtatatctttttatcatctatttgttattttggtataacttaatataagtgtgtcctactttttcactctccatttttttttgtctcttttctttcattacttaaaatgttccatgcaaaatattaaatataacaaattttattacctttttaacactcttaaaaagaaattatttaatatatttagttgactcttctcatttcatttacataagtggatttttttacttcttttatgtaatttaaaataggtaaattgttcagagttcaaaataaatgttttgaatttttccttttttttgacttttatttaaatttttaggttataatttcaagatgtatatatttatagttttactttgaattatttatattttaaaaatagtataaaaggataaaattgaaaaattatgtttaaactttttttaaagaaaatatttattacttcacaagtttacttaatataaaataaagaaagtaacatctatcgacttccttgtgtctagtaaataacacaaggaagtgatagtatatacgaaaaagaaattccatttgtataaaggagtacttctctttgaaatgcatcttacactttcctaattcaatttaatcaagattcaatatatttacgagattcaataaaaattagaaaagtaaaagtaaatgcatgctcttattactcacgggataactttgtccatcttgtttttgtacaaaacgattctttaagaggtcattttttattaaggatacacaataattattttagacaatgtgaaatctctctcaatcaattattccatctcgatgacatataaccccataatatttaaggaaacataattaatttatttgtcttactttatttttgcgttcgaccaagaattggacaagtaggttgggagatagggtcaactaaggcacaaaaagggaaggcaaagagagaaatttgcttcattttctctacaaaaattaatactaatggatacttcaacttctaacagtcaaacaaattcctaacatattacttactgtaatgctataacgtgtatgaaacacaaaaatacagaaaggggttacgtcattatggcctttggcttttgccttttgccagctactactatattattaattcctagttgcagttagcagtttcaagggttgtccgtagcagtcaaatttattcattaatttaacaaaaagatccaatttttatattttttacgatctcattctatataagttccaatctttttgcaagatcttttcagaaaaggaaaaaaggccttttttactttctgggtaggtggataagaactcttatctttgaagggtttttttttttttttattgttttagagagaaaagaggaaatggggtcttttggaatgcttgctagaagcccggggag

SEQ ID NO: 63 - DNA, 27 bp, Artificial Sequence
  Sense nucleotide
tctgttcctcattaatattctgatttt

SEQ ID NO: 64 - DNA, 33 bp, Artificial Sequence
  Antisense nucleotide
ctccccgggcttctagcaagcattccaaaagac

SEQ ID NO: 65 - DNA, 22 bp, Artificial Sequence
  Sense nucleotide
ttgctagaagggctgtgcttac

SEQ ID NO: 66 - DNA, 22 bp, Artificial Sequence
  Antisense nucleotide
gcaccatagcgactaactgaag

SEQ ID NO: 67 - DNA, 20 bp, Artificial Sequence
  Sense nucleotide
aagtggttgccttcccttgc

SEQ ID NO: 68 - DNA, 24 bp, Artificial Sequence
  Antisense nucleotide
gttttgtctctggtttcttctgcc

SEQ ID NO: 69 - DNA, 24 bp, Artificial Sequence
  Synthetic
tggagccacccgcagttcgaaaag

SEQ ID NO: 70 - DNA, 28 bp, Artificial Sequence
  Sense nucleotide
ctctctagatttgtttcccaaataacga

SEQ ID NO: 71 - DNA, 29 bp, Artificial Sequence
  Antisense nucleotide
ctccccgggtcgattgcaaaacacaacaa

SEQ ID NO: 72 - DNA, 2313 bp, Artificial Sequence
  PCR product
ctctctagatttgtttcccaaataacgataaataaataaataaatatcctctccatccaattgatcattacttgtttattactctctctgtctcattttaattaaacttgtgagattaatatatacatattaaaaaaaatattcgaagacaaaatttatatcatacttttcactattgcccttcgtaaaatcataaatatatagtgtaacttatctcttagaaaatataaaagtttaataaataaaagggcaaaaataaaaaaaatctcaaacattcatcctgaactttgaacaattcaattattttgaaccttgaaaaaaagttttaaaactttgtaaatatatattactacttatagattgattaataatatatgtttagcctagaaaattaataaattatttatttgttgtttgtatctattctatttttattattatataatactattcaatatttcatatattttctaccacatttgtattaaatatattcaaaggataatattatctttactattatttattgtttaaataaagtgtgtccaaattaaggtgaataactgttgttagacgtagaaattaaataccccacaaggtatccatactgatatcactttttttttaattagatatctattatttgaatgaatatgacaagaatcttctcctttaaaatcaaatttaaattaattgagattttgatatatagtgaattaaatatgaaattaaaaaataaaagtcaatacgagcccttagatcgaagaagtactagggggaggtgattagacatgatatgccgaaatttaatctcattgaggacatgaccctagataggtagacgtagaggtcgcgaattagaatagtaggataattggttggtagggttaggtggttacctagtcagggggcctaacagggttgagtagtaatatttttttttctagcatgagttgtcattatttgttgcttatatgttaattgtattatatttttgtattatcatgtgctttcttttacttttgtcatatctagtcctttctgagtatggattttaaaatgagggttcccagaaacagtctctctacttaggcagtgataaggtctgcatacattctaccctccctagactccacttatgagattttactgattatattgttgttgttgttgatataattttatttattctattcatgtaccaaaagattcctgaagagatcattttataagaaataacaataataatgaaataactttataaatatgagataattttatctttttccaaccaaacaacccataaatttagggaaacatttactccggaaatataataattactccatcaattttaatttatttatcatatatttttttaaaaactatttttatatatttttttcatttcattttatgtgacacacacatatttaaaaaaaacttttaaaattttatggtttaaaatcgctcttaaatatttgtattgctgaaaattatttcattaaaaataaaatataaaaataaactatttctaattttaataagataatatttttctaagacaatgaataaaaatttagaaagccttcattattttcttaaatcctattaaaataggataacagaaactgaggttgtagaacattttaggggttgaatttgatgaattggacagtaggtgggggatagggcaagaaggcagcaaaaagggtgagaaaaacagaaagaaagaaaggcatacagagaatttcccccttttttttctcttaccaaaattaatggacaattcaacttctaacagtcaaacaaattcctaacatatgcagctataacgtggataaagcagaaaaatacaaaaaaaaggtttccatctttttggcatttgcctttgccagctattactatattattaattcccagttgcagttagcagtttcaagggttgtccgtagcagtcaaatttattcatatttaacaaaaagatccaatttttatattttttacaatccctttatataggttccaagctttttgtaagattttcagaaagggaaaggccttttttgctctgtgggtaggtggataagaactcttttcttgaaggtagtgtttattttattgtttttactgagaaagaggaaatgggttctttcggaatgctcgctagaagagctgttcttaccgatacaccagttatggttcaggtaaattacaagatcctagattggatttcttgctcttttgtttggtttaaggttctgtgctttaatgggatatgttgttgttgtgttttgcaatcgacccggggag

SEQ ID NO: 73 - DNA, 1209 bp, Artificial Sequence
  Sequence based on Solanum melongena cDNA
atgggttctttcggaatgctcgctagaagagctgttcttaccgatacaccagttatggttcagatacaagaactgattcgaggtaataaagattgtatttctctagctcagggagtagtgtactggcaaccacctgcacaagcacttgaaaaggtgaaagaaattatctgggaaccttcagttagtcgctatggtgctgatgagggccttcctgagcttagggaggcgttgatgcaaaagttgggtcatgaaaataacctccataaatcctcggtgatggttactgctggtgctaatcaggctttcgtaaatgtcgttctcaccctgtgtgatgctggtgattcagttgttatgtttgcaccatactatttcaatgcacacatgtcattccagatgacaggtgttactgatattctggtgggtcctggtgatcccaagacactccatcctgatgcagactggttggagagtactttaaagaatactgtaccaacaccaaagctcgtcactgttgttaatcctggcaatccatcaggaacatatatccccgagtctcttcttaagaggatatctgatatttgtaagaaggcaggatgttggctcgtaattgataacacatatgagtatttcatgtatgataatcggaaacatgtttgcatagaagcaaaccacattgtcaacatcttttccttctctaaagcatatgggatgatgggatggagagttggatatatagcatacccatcggaagtggaagggcttgcagctcaactccttaaagttcaggacaacataccaatctgtgcttcaataatctcacaacgactggctctttactcaatggaaatgggaccagaatgggtaactaatcaagtaaaagaccttgtcaagaacagagaggtgcttctagaagccttatctcctttgggaaagggagctgttaaagggggagaaggtgccatttacctgtgggcaaagctgccagataaatacatggacgacttcaaagtagttcactggctagctaagaggcatggagtagtcctgatccctggaagttccagcggttgtccaggttatgttagggtctcctttggaggattgatcgagaaggactgtcgagcagctgcagaaaggctcagaaaaggtttggaagagctggtaaatagtggaatggcgtcatggagccacccgcagttcgaaaagtga

SEQ ID NO: 74 - DNA, 1209 bp, Artificial Sequence
  Sequence based on Solanum melongena cDNA
atggggtcctttggcatgctagcgcgtcgtgcagtgttgaccgataccccggtcatggttcagattcaggagttgatccgcggtaacaaagattgcattagcctcgctcaaggggtagtgtattggcaacctccagcacaagcgttggaaaaggtgaaggagatcatctgggagccgagtgtgagccgctatggtgcggatgaaggactgccggaactgcgtgaagccctgatgcaaaaactcggccacgaaaacaatctgcacaaaagctcagtgatggtgacggcaggtgcaaatcaggcgtttgttaatgtggtcctgacactgtgtgatgcaggtgactctgtggtcatgtttgcgccgtactactttaacgcccacatgagcttccagatgactggcgtaaccgacatcctggtaggtccaggtgaccccaaaacgctgcatcctgatgcggattggctcgaatcgacgctgaaaaacacagttcccaccccgaaacttgtcactgttgtcaatccgggtaatccgagtggcacgtacattccggaaagtctgttaaaacggatttccgacatctgcaaaaaagccggctgttggttggtgatagataacacctatgagtactttatgtatgacaatcgcaaacatgtgtgcattgaagcgaaccacattgtaaacatcttctcgttctcaaaggcgtatggtatgatgggctggagagttggatatatcgcctatccgtcggaagtggaagggttagccgcacaactgcttaaagtccaggataacattcccatatgcgcttctatcatttcccagcgtttagccctgtactccatggaaatgggaccagagtgggtgaccaaccaggtcaaggatctggtaaaaaatcgcgaagttctgcttgaagcgttgtctcctctcggaaaaggcgccgttaagggcggggaaggtgcgatttacctgtgggctaaactgccggataagtatatggacgacttcaaagttgtccattggctggcgaaacgtcatggcgtggttctgattccgggtagcagctcaggctgtccaggctatgtgcgcgtttcgtttggcgggttaatcgagaaagattgtcgtgctgcagctgaacgacttcgcaaaggcctggaagagttagtaaatagcggtatggccagttggtctcatccgcagttcgaaaaataa

SEQ ID NO: 75 - DNA, 16 bp, Artificial Sequence
  Synthetic nucleotide
taccatggcgggatcc

SEQ ID NO: 76 - DNA, 17 bp, Artificial Sequence
  Synthetic nucleotide
taggccgcataagcccg

SEQ ID NO: 77 - DNA, 1242 bp, Artificial Sequence
  Synthetic sequence
taccatggcgggatccatggggtcctttggcatgctagcgcgtcgtgcagtgttgaccgataccccggtcatggttcagattcaggagttgatccgcggtaacaaagattgcattagcctcgctcaaggggtagtgtattggcaacctccagcacaagcgttggaaaaggtgaaggagatcatctgggagccgagtgtgagccgctatggtgcggatgaaggactgccggaactgcgtgaagccctgatgcaaaaactcggccacgaaaacaatctgcacaaaagctcagtgatggtgacggcaggtgcaaatcaggcgtttgttaatgtggtcctgacactgtgtgatgcaggtgactctgtggtcatgtttgcgccgtactactttaacgcccacatgagcttccagatgactggcgtaaccgacatcctggtaggtccaggtgaccccaaaacgctgcatcctgatgcggattggctcgaatcgacgctgaaaaacacagttcccaccccgaaacttgtcactgttgtcaatccgggtaatccgagtggcacgtacattccggaaagtctgttaaaacggatttccgacatctgcaaaaaagccggctgttggttggtgatagataacacctatgagtactttatgtatgacaatcgcaaacatgtgtgcattgaagcgaaccacattgtaaacatcttctcgttctcaaaggcgtatggtatgatgggctggagagttggatatatcgcctatccgtcggaagtggaagggttagccgcacaactgcttaaagtccaggataacattcccatatgcgcttctatcatttcccagcgtttagccctgtactccatggaaatgggaccagagtgggtgaccaaccaggtcaaggatctggtaaaaaatcgcgaagttctgcttgaagcgttgtctcctctcggaaaaggcgccgttaagggcggggaaggtgcgatttacctgtgggctaaactgccggataagtatatggacgacttcaaagttgtccattggctggcgaaacgtcatggcgtggttctgattccgggtagcagctcaggctgtccaggctatgtgcgcgtttcgtttggcgggttaatcgagaaagattgtcgtgctgcagctgaacgacttcgcaaaggcctggaagagttagtaaatagcggtatggccagttggtctcatccgcagttcgaaaaataataggccgcataagcccg

SEQ ID NO: 78 - protein, 7 aa, Artificial sequence
  Sequence from expression vector
TSTMAGS